European Patent Application EP 4 354 139 A1, published April 17, 2024. Title: NON-INVASIVE METHOD OF CELL IMAGING. Applicant: Fundación Carlos Simón para la Investigación en Salud de la Mujer. The sequence listing filed with the application follows.

SEQUENCE LISTING (4 sequences)

SEQ ID NO: 1 - DNA, 21 bp, synthetic construct
  source 1..21: mol_type = other DNA
aaccatgtaccagattaagta

SEQ ID NO: 2 - DNA, 21 bp, synthetic construct
  source 1..21: mol_type = other DNA
atggatggcatcatcgctgaa

SEQ ID NO: 3 - DNA, 21 bp, synthetic construct
  source 1..21: mol_type = other DNA
cagagtggtgtccgagactaa

SEQ ID NO: 4 - DNA, 21 bp, synthetic construct
  source 1..21: mol_type = other DNA
ccgggaacatctggagaagaa